European Patent Application EP 4 631 971 A1, published October 15, 2025. Title: A novel Mn-dependent transcriptional regulator variant and preparation method of L-amino acid using thereof. Applicant: CJ CheilJedang Corporation. The sequence listing filed with the application follows.

SEQUENCE LISTING (8 sequences)

SEQ ID NO: 1 - protein, 239 aa, unidentified
LSLEKQGRQPPVKDLVDTTEMYLRTIYELEEEGIVPLRARIAERLEQSGPTVSQTVARMERDGLVHVSPDRSLEMTPEGRSLAIAVMRKHRLAERLLTDIIGLDIHKVHDEACRWEHVMSDEVERRLVEVLDDVHRSPFGNPIPGLGEIGLDQADEPDSGVRAIDLPLGENLKARIVQLNEILQVDLEQFQALTDAGVEIGTEVDIINEQGRVVITHNGSSVELIDDLAHAVRVEKVEG

SEQ ID NO: 2 - DNA, 720 bp, unidentified
  source 1..720: mol_type = genomic DNA
ttgagtttggaaaaacaaggaaggcagcctcctgtgaaggatctggtcgataccaccgaaatgtatctgcgcactatttacgagctggaagaagagggcattgttcctctgcgtgctcgtatcgcagaacgccttgagcagtccggcccaactgtcagccagactgtcgcccgtatggaacgcgacggtcttgtgcacgtcagccccgaccgcagcctcgaaatgactccagagggacgttccctcgccatcgccgtgatgcgtaagcaccgcctagcagaacgcctccttaccgacatcatcggcttggacatccacaaagtccacgacgaagcatgccgctgggagcacgtgatgagtgatgaggttgaacgtcgcctcgttgaagttcttgacgatgtgcatcgctcccctttcggtaacccaattcctggcctcggcgaaatcggtttggatcaagcagatgagcctgattccggcgttcgtgccatcgatctgcctctcggtgagaacctgaaggctcgcatcgtacagctcaacgagatcctgcaggtagatcttgagcagttccaggcactcaccgacgcgggtgttgaaatcggtaccgaagtagacatcatcaatgagcagggccgggtcgtgatcacccacaacggctccagcgtagaactgattgacgatcttgcacatgcagtccgcgtagaaaaggttgagggctaa

SEQ ID NO: 3 - protein, 239 aa, synthetic construct
LSLEKQGRQPPVKDLVDTTEMYLRTIYELEEEGIVPLRARIAERLEQSGPTVSQTVARMERDGLVHVSPDRSLEMTPEGRSLAIAVMRKHRLAERLLTDIIGLDIHKVHDEACRWEHVMSDEVERRLVEVLDDVHRSPFGNPIPGLGEIGLDQADEPDSDVRAIDLPLGENLKARIVQLNEILQVDLEQFQALTDAGVEIGTEVDIINEQGRVVITHNGSSVELIDDLAHAVRVEKVEG

SEQ ID NO: 4 - DNA, 720 bp, synthetic construct
  source 1..720: mol_type = other DNA
ttgagtttggaaaaacaaggaaggcagcctcctgtgaaggatctggtcgataccaccgaaatgtatctgcgcactatttacgagctggaagaagagggcattgttcctctgcgtgctcgtatcgcagaacgccttgagcagtccggcccaactgtcagccagactgtcgcccgtatggaacgcgacggtcttgtgcacgtcagccccgaccgcagcctcgaaatgactccagagggacgttccctcgccatcgccgtgatgcgtaagcaccgcctagcagaacgcctccttaccgacatcatcggcttggacatccacaaagtccacgacgaagcatgccgctgggagcacgtgatgagtgatgaggttgaacgtcgcctcgttgaagttcttgacgatgtgcatcgctcccctttcggtaacccaattcctggcctcggcgaaatcggtttggatcaagcagatgagcctgattccgacgttcgtgccatcgatctgcctctcggtgagaacctgaaggctcgcatcgtacagctcaacgagatcctgcaggtagatcttgagcagttccaggcactcaccgacgcgggtgttgaaatcggtaccgaagtagacatcatcaatgagcagggccgggtcgtgatcacccacaacggctccagcgtagaactgattgacgatcttgcacatgcagtccgcgtagaaaaggttgagggctaa

SEQ ID NO: 5 - DNA, 33 bp, synthetic construct
  source 1..33: mol_type = other DNA
cggtacccggggatccgcataaattgagtttgg

SEQ ID NO: 6 - DNA, 35 bp, synthetic construct
  source 1..35: mol_type = other DNA
atcgatggcacgaacgtcggaatcaggctcatctg

SEQ ID NO: 7 - DNA, 35 bp, synthetic construct
  source 1..35: mol_type = other DNA
acgttcgtgccatcgatctgcctctcggtgagaac

SEQ ID NO: 8 - DNA, 35 bp, synthetic construct
  source 1..35: mol_type = other DNA
atgcctgcaggtcgacgggcttttccactgattcg